European Patent Specification EP 3 677 593 B1, published August 7, 2024. Title: A modified HSV gB protein and a vaccine comprising the same. Applicant: KM Biologics Co., Ltd. The sequence listing filed with the application follows.

SEQUENCE LISTING (4 sequences)

SEQ ID NO: 1 - protein, 705 aa, Herpes simplex virus-2
  HSV gB1-705
APAAPAAPRASGGVAATVAANGGPASRPPPVPSPATTKARKRKTKKPPKRPEATPPPDANATVAAGHATLRAHLREIKVENADAQFYVCPPPTGATVVQFEQPRRCPTRPEGQNYTEGIAVVFKENIAPYKFKATMYYKDVTVSQVWFGHRYSQFMGIFEDRAPVPFEEVIDKINAKGVCRSTAKYVRNNMETTAFHRDDHETDMELKPAKVATRTSRGWHTTDLKYNPSRVEAFHRYGTTVNCIVEEVDARSVYPYDEFVLATGDFVYMSPFYGYREGSHTEHTSYAADRFKQVDGFYARDLTTKARATSPTTRNLLTTPKFTVAWDWVPKRPAVCTMTKWQEVDEMLRAEYGGSFRFSSDAISTTFTTNLTQYSLSRVDLGDCIGRDAREAIDRMFARKYNATHIKVGQPQYYLATGGFLIAYQPLLSNTLAELYVREYMREQDRKPRNATPAPLREAPSANASVERIKTTSSIEFARLQFTYNHIQRHVNDMLGRIAVAWCELQNHELTLWNEARKLNPNAIASATVGRRVSARMLGDVMAVSTCVPVAPDNVIVQNSMRVSSRPGTCYSRPLVSFRYEDQGPLIEGQLGENNELRLTRDALEPCTVGHRRYFIFGGGYVYFEEYAYSHQLSRADVTTVSTFIDLNITMLEDHEFVPLEVYTRHEIKDSGLLDYTEVQRRNQLHDLRFADIDTVIRADANAA

SEQ ID NO: 2 - protein, 904 aa, Herpes simplex virus-1
MHQGAPSWGRRWFVVWALLGLTLGVLVASAAPTSPGTPGVAAATQAANGGPATPAPPPLGAAPTGDPKPKKNKKPKNPTPPRPAGDNATVAAGHATLREHLRDIKAENTDANFYVCPPPTGATVVQFEQPRRCPTRPEGQNYTEGIAVVFKENIAPYKFKATMYYKDVTVSQVWFGHRYSQFMGIFEDRAPVPFEEVIDKINAKGVCRSTAKYVRNNLETTAFHRDDHETDMELKPANAATRTSRGWHTTDLKYNPSRVEAFHRYGTTVNCIVEEVDARSVYPYDEFVLATGDFVYMSPFYGYREGSHTEHTTYAADRFKQVDGFYARDLTTKARATAPTTRNLLTTPKFTVAWDWVPKRPSVCTMTKWQEVDEMLRSEYGGSFRFSSDAISTTFTTNLTEYPLSRVDLGDCIGKDARDAMDRIFARRYNATHIKVGQPQYYQANGGFLIAYQPLLSNTLAELYVREHLREQSRKPPNPTPPPPGASANASVERIKTTSSIEFARLQFTYNHIQRHVNDMLGRVAIAWCELQNHELTLWNEARKLNPNAIASVTVGRRVSARMLGDVMAVSTCVPVAADNVIVQNSMRISSRPGACYSRPLVSFRYEDQGPLVEGQLGENNELRLTRDAIEPCTVGHRRYFTFGGGYVYFEEYAYSHQLSRADITTVSTFIDLNITMLEDHEFVPLEVYTRHEIKDSGLLDYTEVQRRNQLHDLRFADIDTVIHADANAAMFAGLGAFFEGMGDLGRAVGKVVMGIVGGVVSAVSGVSSFMSNPFGALAVGLLVLAGLAAAFFAFRYVMRLQSNPMKALYPLTTKELKNPTNPDASGEGEEGGDFDEAKLAEAREMIRYMALVSAMERTEHKAKKKGTSALLSAKVTDMVMRKRRNTNYTQVPNKDGDADEDDL

SEQ ID NO: 3 - protein, 946 aa, Herpes simplex virus-2
MRGGGLICALVVGALVAAVASAAPAAPAAPRASGGVAATVAANGGPASRPPPVPSPATTKARKRKTKKPPKRPEATPPPDANATVAAGHATLRAHLREIKVENADAQFYVCPPPTGATVVQFEQPRRCPTRPEGQNYTEGIAVVFKENIAPYKFKATMYYKDVTVSQVWFGHRYSQFMGIFEDRAPVPFEEVIDKINAKGVCRSTAKYVRNNMETTAFHRDDHETDMELKPAKVATRTSRGWHTTDLKYNPSRVEAFHRYGTTVNCIVEEVDARSVYPYDEFVLATGDFVYMSPFYGYREGSHTEHTSYAADRFKQVDGFYARDLTTKARATSPTTRNLLTTPKFTVAWDWVPKRPAVCTMTKWQEVDEMLRAEYGGSFRFSSDAISTTFTTNLTQYSLSRVDLGDCIGRDAREAIDRMFARKYNATHIKVGQPQYYLATGGFLIAYQPLLSNTLAELYVREYMREQDRKPRNATPAPLREAPSANASVERIKTTSSIEFARLQFTYNHIQRHVNDMLGRIAVAWCELQNHELTLWNEARKLNPNAIASATVGRRVSARMLGDVMAVSTCVPVAPDNVIVQNSMRVSSRPGTCYSRPLVSFRYEDQGPLIEGQLGENNELRLTRDALEPCTVGHRRYFIFGGGYVYFEEYAYSHQLSRADVTTVSTFIDLNITMLEDHEFVPLEVYTRHEIKDSGLLDYTEVQRRNQLHDLRFADIDTVIRADANAAMFAGLCAFFEGMGDLGRAVGKVVMGVVGGVVSAVSGVSSFMSNPFGALAVGLLVLAGLVAAFFAFRYVLQLQRNPMKALYPLTTKELKTSDPGGVGGEGEEGAEGGGFDEAKLAEAREMIRYMALVSAMERTEHKARKKGTSALLSSKVTNMVLRKRNKARYSPLHNEDEAGDEDELARKKGTSALLSSKVTNMVLRKRNKARYSPLHNEDEAGDEDEL

SEQ ID NO: 4 - DNA, 2712 bp, Herpes simplex virus-2
atgcgcggggggggcttgatttgcgcgctggtcgtgggggcgctggtggccgcggtggcgtcggcggccccggcggccccggcggccccccgcgcctcgggcggcgtggccgcgaccgtcgcggcgaacgggggtcccgcctcccggccgccccccgtcccgagccccgcgaccaccaaggcccggaagcggaaaaccaaaaagccgcccaagcggcccgaggcgaccccgccccccgacgccaacgcgaccgtcgccgccggccacgccacgctgcgcgcgcacctgcgggaaatcaaggtcgagaacgccgatgcccagttttacgtgtgcccgcccccgacgggcgccacggtggtgcagtttgagcagccgcgccgctgcccgacgcgcccggaggggcagaactacacggagggcatcgcggtggtcttcaaggagaacatcgccccgtacaaattcaaggccaccatgtactacaaagacgtgaccgtgtcgcaggtgtggttcggccaccgctactcccagtttatggggatattcgaggaccgcgcccccgttcccttcgaggaggtgatcgacaagattaacgccaagggggtctgccgctccacggccaagtacgtgcggaacaacatggagaccaccgcgtttcaccgggacgaccacgagaccgacatggagctcaagccggcgaaggtcgccacgcgcacgagccgggggtggcacaccaccgacctcaagtacaacccctcgcgggtggaggcgttccatcggtacggcacgacggtcaactgcatcgtcgaggaggtggacgcgcggtcggtgtacccgtacgatgagtttgtgttggcgacgggcgactttgtgtacatgtccccgttttacggctaccgggaggggtcgcacaccgagcacaccagctacgccgccgaccgcttcaagcaggtcgacggcttctacgcgcgcgacctcaccacgaaggcccgggccacgtcgccgacgacccgcaacttgctgacgacccccaagtttaccgtggcctgggactgggtgccgaagcgaccggcggtctgcaccatgaccaagtggcaggaggtggacgagatgctccgcgccgagtacggcggctccttccgcttctcctccgacgccatctcgaccaccttcaccaccaacctgacccagtactcgctctcgcgcgtcgacctgggcgactgcattggccgggatgcccgcgaggccatcgaccgcatgtttgcgcgcaagtacaacgccacgcacatcaaggtgggccagccgcagtactacctggccacggggggcttcctcatcgcgtaccagcccctcctcagcaacacgctcgccgagctgtacgtgcgggagtacatgcgggagcaggaccgcaagccccggaatgccacgcccgcgccactgcgggaggcgcccagcgccaacgcgtccgtggagcgcatcaagaccacctcctcgatcgagttcgcccggctgcagtttacgtataaccacatacagcgccacgtgaacgacatgctggggcgcatcgccgtcgcgtggtgcgagctgcagaaccacgagctgactctctggaacgaggcccgcaagctcaaccccaacgccatcgcctccgccaccgtcggccggcgggtgagcgcgcgcatgctcggagacgtcatggccgtctccacgtgcgtgcccgtcgccccggacaacgtgatcgtgcagaactcgatgcgcgtcagctcgcggccggggacgtgctacagccgccccctggtcagctttcggtacgaagaccagggcccgctgatcgaggggcagctgggcgagaacaacgagctgcgcctcacccgcgacgcgctcgagccgtgcaccgtgggccaccggcgctacttcatcttcggcgggggctacgtgtacttcgaggagtacgcgtactctcaccagctgagtcgcgccgacgtcaccaccgtcagcaccttcatcgacctgaacatcaccatgctggaggaccacgagtttgtgcccctggaggtctacacgcgccacgagatcaaggacagcggcctgctggactacacggaggtccagcgccgcaaccagctgcacgacctgcgctttgccgacatcgacacggtcatccgcgccgacgccaacgccgccatgttcgcggggctgtgcgcgttcttcgaggggatgggggacttggggcgcgcggtcggcaaggtagtcatgggagtagtggggggcgtggtgtcggccgtctcgggcgtgtcctcctttatgtccaaccccttcggggcgcttgccgtggggctgctggtcctggccggcctggtcgcggccttcttcgccttccgctacgtcctgcaactgcaacgcaatcccatgaaggccctgtatccgctcaccaccaaggaactcaagacttccgaccccgggggcgtgggcggggagggggaggaaggcgcggaggggggcgggtttgacgaggccaagttggccgaggcccgagaaatgatccgatatatggctttggtgtcggccatggagcgcacggaacacaaggccagaaagaagggcacgagcgccctgctcagctccaaggtcaccaacatggttctgcgcaagcgcaacaaagccaggtactctccgctccacaacgaggacgaggccggagacgaagacgagctc